European Patent Application EP 4 279 508 A1, published November 22, 2023. Title: FULLY HUMAN ANTIBODY TARGETING CD5. Applicant: Nanjing IASO Biotherapeutics Co., Ltd. The sequence listing filed with the application follows.

SEQUENCE LISTING (21 sequences)

SEQ ID NO: 1 - protein, 8 aa, Artificial Sequence
  #42 HCDR1 amino acid sequence
GFTFSHSA

SEQ ID NO: 2 - protein, 8 aa, Artificial Sequence
  #42 HCDR2 amino acid sequence
IYARGGYT

SEQ ID NO: 3 - protein, 14 aa, Artificial Sequence
  #42 HCDR3 amino acid sequence
ARGYHLEYMVSQDV

SEQ ID NO: 4 - protein, 8 aa, Artificial Sequence
  #60 HCDR1 amino acid sequence
GFTFSSYE

SEQ ID NO: 5 - protein, 8 aa, Artificial Sequence
  #60 HCDR2 amino acid sequence
ISSSGSTI

SEQ ID NO: 6 - protein, 10 aa, Artificial Sequence
  #60 HCDR3 amino acid sequence
ARVAQREGDV

SEQ ID NO: 7 - protein, 8 aa, Artificial Sequence
  #61 HCDR1 amino acid sequence
GGTFSNYA

SEQ ID NO: 8 - protein, 8 aa, Artificial Sequence
  #61 HCDR2 amino acid sequence
ISAYNGDT

SEQ ID NO: 9 - protein, 11 aa, Artificial Sequence
  #61 HCDR3 amino acid sequence
ARYESMSGQDI

SEQ ID NO: 10 - protein, 8 aa, Artificial Sequence
  #62 HCDR1 amino acid sequence
GYSFSNHW

SEQ ID NO: 11 - protein, 8 aa, Artificial Sequence
  #62 HCDR2 amino acid sequence
VYPGDSDT

SEQ ID NO: 12 - protein, 16 aa, Artificial Sequence
  #62 HCDR3 amino acid sequence
ARGGTIDGDYGGRQDF

SEQ ID NO: 13 - DNA, 363 bp, Artificial Sequence
  #42 VH DNA sequence
gaagttcagctgctggaaagcggtggtggtctggttcagcctggtggtagcctgcgtctgagctgtgcagcaagcggttttacctttagccatagcgccatgggttgggttcgtcaggcacctggtaaaggtctggaatgggttagcagcatctatgcccgcggcggctatacctattatgcagatagcgttaaaggtcgttttaccattagccgtgataacagcaaaaataccctgtacctgcagatgaatagtctgcgtgcagaggataccgcagtgtattattgtgcgcgcggttaccatctggaatacatggtttctcaggatgtttggggtcaaggtactctggtgaccgtctcctca

SEQ ID NO: 14 - DNA, 351 bp, Artificial Sequence
  #60 VH DNA sequence
caggtgcagctggtggagtctgggggaggcttggtacagcctggagggtccctgagactctcctgtgcagcctctggattcaccttcagtagttatgaaatgaactgggtccgccaggctccagggaaggggctggagtgggtttcatacattagtagtagtggtagtaccatatactacgcagactctgtgaagggccgattcaccatctccagagacaacgccaagaactcactgtatctgcaaatgaacagtctgagagccgaggacacggctgtttattactgtgcgagagtcgcccagagagaaggggacgtctggggcaaagggaccacggtcaccgtctcctca

SEQ ID NO: 15 - DNA, 354 bp, Artificial Sequence
  #61 VH DNA sequence
caggtgcagctggtgcagtctggggctgaggtgaagaagcctgggtcctcggtgaaggtctcctgcaaggcttctggaggcaccttcagcaactatgctatcagctgggtgcgacaggcccctggacaagggcttgagtggatgggatggatcagcgcctacaatggtgacacaaaatatgcacagaggctccagggcagagtcaccatgaccacagacacatccacgagcacagcctacatggagctgaggaacctaagatctgacgacacggccgtgtattactgtgcgcgctacgaatctatgtctggtcaggatatctggggtcaaggtactctggtgaccgtctcctca

SEQ ID NO: 16 - DNA, 369 bp, Artificial Sequence
  #62 VH DNA sequence
caggtccagctggtgcagtctggggctgaggtgaaaaagcccggggagtctctgaggatctcctgtaaggcttctggatacagttttagcaaccattggatcggctgggtgcgccagaagcccgggaaaggcctggagtggatggggagcgtctatcctggtgactccgataccagatacagcccgtccttccaaggccacgtcactgtctcagccgacaagtccatgaataccgcctacctgcagtggagcagcctgaagacctcggacaccgccatgtattattgtgcgagaggtgggactattgacggtgactacggggggaggcaagacttctggggccagggaaccatggtcaccgtctcttca

SEQ ID NO: 17 - protein, 121 aa, Artificial Sequence
  #42 VH amino acid sequence
EVQLLESGGGLVQPGGSLRLSCAASGFTFSHSAMGWVRQAPGKGLEWVSSIYARGGYTYYADSVKGRFTISRDNSKNTLYLQMNSLRAEDTAVYYCARGYHLEYMVSQDVWGQGTLVTVSS

SEQ ID NO: 18 - protein, 117 aa, Artificial Sequence
  #60 VH amino acid sequence
QVQLVESGGGLVQPGGSLRLSCAASGFTFSSYEMNWVRQAPGKGLEWVSYISSSGSTIYYADSVKGRFTISRDNAKNSLYLQMNSLRAEDTAVYYCARVAQREGDVWGKGTTVTVSS

SEQ ID NO: 19 - protein, 118 aa, Artificial Sequence
  #61 VH amino acid sequence
QVQLVQSGAEVKKPGSSVKVSCKASGGTFSNYAISWVRQAPGQGLEWMGWISAYNGDTKYAQRLQGRVTMTTDTSTSTAYMELRNLRSDDTAVYYCARYESMSGQDIWGQGTLVTVSS

SEQ ID NO: 20 - protein, 123 aa, Artificial Sequence
  #62 VH amino acid sequence
QVQLVQSGAEVKKPGESLRISCKASGYSFSNHWIGWVRQKPGKGLEWMGSVYPGDSDTRYSPSFQGHVTVSADKSMNTAYLQWSSLKTSDTAMYYCARGGTIDGDYGGRQDFWGQGTMVTVSS

SEQ ID NO: 21 - protein, 15 aa, Artificial Sequence
  Linker sequence
GGGGSGGGGSGGGGS